European Patent Application EP 4 353 736 A1, published April 17, 2024. Title: Bio PROTAC Protein having Intracellular Delevery Function and Pharmaceutical Composition Comprising the Same. Applicant: NIBEC Co., Ltd. Seoul National University R&DB Foundation. The sequence listing filed with the application follows.

SEQUENCE LISTING (24 sequences)

SEQ ID NO: 1 - protein, 485 aa, Artificial Sequence
  chimera protein
EVQLLESGGGLVQPGGSLRLSCAASGFTFSTFSMNWVRQAPGKGLEWVSYISRTSKTIYYADSVKGRFTISRDNSKNTLYLQMNSLRAEDTAVYYCARGRFFDYWGQGTLVTVSSGGSEGKSSGSGSESKSTGGSDIQMTQSPSSLSASVGDRVTITCRASQSISSYLNWYQQKPGEAPKLLIYSASVLQSGVPSRFSGSGSGTDFTLTISSLQPEDFATYYCQQSVMIPMTFGQGTKVEIKGSGGGGSMPRRAENWDEAEVGAEEAGVEEYGPEEDGGEESGAEESGPEESGPEELGAEEEMEAGRPRPVLRSVNSREPSQVIFCNRSPRVVLPVWLNFDGEPQPYPTLPPGTGRRIHSYRGHLWLFRDAGTHDGLLVNQTELFVPSLNVDGQPIFANITLPVYTLKERCLQVVRSLVKPENYRRLDIVRSLYEDLEDHPNVQKDLERLTQERIAHQRMGDENLYFQGGSGGSGGSHHHHHHHH

SEQ ID NO: 2 - protein, 523 aa, Artificial Sequence
  chimera protein
MAWVWTLLFLMAAAQSIQAVSRRRRRRGGRRRRGGGGSEVQLLESGGGLVQPGGSLRLSCAASGFTFSTFSMNWVRQAPGKGLEWVSYISRTSKTIYYADSVKGRFTISRDNSKNTLYLQMNSLRAEDTAVYYCARGRFFDYWGQGTLVTVSSGGSEGKSSGSGSESKSTGGSDIQMTQSPSSLSASVGDRVTITCRASQSISSYLNWYQQKPGEAPKLLIYSASVLQSGVPSRFSGSGSGTDFTLTISSLQPEDFATYYCQQSVMIPMTFGQGTKVEIKGSGGGGSMPRRAENWDEAEVGAEEAGVEEYGPEEDGGEESGAEESGPEESGPEELGAEEEMEAGRPRPVLRSVNSREPSQVIFCNRSPRVVLPVWLNFDGEPQPYPTLPPGTGRRIHSYRGHLWLFRDAGTHDGLLVNQTELFVPSLNVDGQPIFANITLPVYTLKERCLQVVRSLVKPENYRRLDIVRSLYEDLEDHPNVQKDLERLTQERIAHQRMGDENLYFQGGSGGSGGSHHHHHHHH

SEQ ID NO: 3 - protein, 523 aa, Artificial Sequence
  chimera protein
MAWVWTLLFLMAAAQSIQAEVQLLESGGGLVQPGGSLRLSCAASGFTFSTFSMNWVRQAPGKGLEWVSYISRTSKTIYYADSVKGRFTISRDNSKNTLYLQMNSLRAEDTAVYYCARGRFFDYWGQGTLVTVSSGGSEGKSSGSGSESKSTGGSDIQMTQSPSSLSASVGDRVTITCRASQSISSYLNWYQQKPGEAPKLLIYSASVLQSGVPSRFSGSGSGTDFTLTISSLQPEDFATYYCQQSVMIPMTFGQGTKVEIKGSGGGGSMPRRAENWDEAEVGAEEAGVEEYGPEEDGGEESGAEESGPEESGPEELGAEEEMEAGRPRPVLRSVNSREPSQVIFCNRSPRVVLPVWLNFDGEPQPYPTLPPGTGRRIHSYRGHLWLFRDAGTHDGLLVNQTELFVPSLNVDGQPIFANITLPVYTLKERCLQVVRSLVKPENYRRLDIVRSLYEDLEDHPNVQKDLERLTQERIAHQRMGDGGGGSVSRRRRRRGGRRRRENLYFQGGSGGSGGSHHHHHHHH

SEQ ID NO: 4 - protein, 464 aa, Artificial Sequence
  chimera protein
EVQLLESGGGLVQPGGSLRLSCAASGFTFSTFSMNWVRQAPGKGLEWVSYISRTSKTIYYADSVKGRFTISRDNSKNTLYLQMNSLRAEDTAVYYCARGRFFDYWGQGTLVTVSSGGSEGKSSGSGSESKSTGGSDIQMTQSPSSLSASVGDRVTITCRASQSISSYLNWYQQKPGEAPKLLIYSASVLQSGVPSRFSGSGSGTDFTLTISSLQPEDFATYYCQQSVMIPMTFGQGTKVEIKGSGGGGSMENRWQVMIVWQVDRMRIRTWKSLVKHHMYVSGKARGWFYRHHYESPHPRISSEVHIPLGDARLVITTYWGLHTGERDWHLGQGVSIEWRKKRYSTQVDPELADQLIHLYYFDCFSDSAIRKALLGHIVSPRCEYQAGHNKVGSLQYLALAALITPKKIKPPLPSVTKLTEDRWNKPQKTKGHRGSHTMNGHENLYFQGGSGGSGGSHHHHHHHH

SEQ ID NO: 5 - protein, 502 aa, Artificial Sequence
  chimera protein
MAWVWTLLFLMAAAQSIQAVSRRRRRRGGRRRRGGGGSEVQLLESGGGLVQPGGSLRLSCAASGFTFSTFSMNWVRQAPGKGLEWVSYISRTSKTIYYADSVKGRFTISRDNSKNTLYLQMNSLRAEDTAVYYCARGRFFDYWGQGTLVTVSSGGSEGKSSGSGSESKSTGGSDIQMTQSPSSLSASVGDRVTITCRASQSISSYLNWYQQKPGEAPKLLIYSASVLQSGVPSRFSGSGSGTDFTLTISSLQPEDFATYYCQQSVMIPMTFGQGTKVEIKGSGGGGSMENRWQVMIVWQVDRMRIRTWKSLVKHHMYVSGKARGWFYRHHYESPHPRISSEVHIPLGDARLVITTYWGLHTGERDWHLGQGVSIEWRKKRYSTQVDPELADQLIHLYYFDCFSDSAIRKALLGHIVSPRCEYQAGHNKVGSLQYLALAALITPKKIKPPLPSVTKLTEDRWNKPQKTKGHRGSHTMNGHENLYFQGGSGGSGGSHHHHHHHH

SEQ ID NO: 6 - protein, 502 aa, Artificial Sequence
  chimera protein
MAWVWTLLFLMAAAQSIQAEVQLLESGGGLVQPGGSLRLSCAASGFTFSTFSMNWVRQAPGKGLEWVSYISRTSKTIYYADSVKGRFTISRDNSKNTLYLQMNSLRAEDTAVYYCARGRFFDYWGQGTLVTVSSGGSEGKSSGSGSESKSTGGSDIQMTQSPSSLSASVGDRVTITCRASQSISSYLNWYQQKPGEAPKLLIYSASVLQSGVPSRFSGSGSGTDFTLTISSLQPEDFATYYCQQSVMIPMTFGQGTKVEIKGSGGGGSMENRWQVMIVWQVDRMRIRTWKSLVKHHMYVSGKARGWFYRHHYESPHPRISSEVHIPLGDARLVITTYWGLHTGERDWHLGQGVSIEWRKKRYSTQVDPELADQLIHLYYFDCFSDSAIRKALLGHIVSPRCEYQAGHNKVGSLQYLALAALITPKKIKPPLPSVTKLTEDRWNKPQKTKGHRGSHTMNGHGGGGSVSRRRRRRGGRRRRENLYFQGGSGGSGGSHHHHHHHH

SEQ ID NO: 7 - protein, 12 aa, Artificial Sequence
  binder that binds to the RAS superfamily
LTPHKHHKHLHA

SEQ ID NO: 8 - protein, 12 aa, Artificial Sequence
  binder that binds to the RAS superfamily
WPGKHHNHYLRS

SEQ ID NO: 9 - protein, 12 aa, Artificial Sequence
  binder that binds to the RAS superfamily
HDGYWWHSMTMW

SEQ ID NO: 10 - protein, 12 aa, Artificial Sequence
  binder that binds to the RAS superfamily
LIHPMTVKHVHL

SEQ ID NO: 11 - protein, 12 aa, Artificial Sequence
  binder that binds to the RAS superfamily
GSHWHFPKHQQQ

SEQ ID NO: 12 - protein, 12 aa, Artificial Sequence
  binder that binds to the RAS superfamily
GSHWHFPKHQQH

SEQ ID NO: 13 - protein, 12 aa, Artificial Sequence
  binder that binds to the RAS superfamily
WPGKHHHHYLRR

SEQ ID NO: 14 - protein, 242 aa, Artificial Sequence
  binder that binds to the RAS superfamily
EVQLLESGGGLVQPGGSLRLSCAASGFTFSTFSMNWVRQAPGKGLEWVSYISRTSKTIYYADSVKGRFTISRDNSKNTLYLQMNSLRAEDTAVYYCARGRFFDYWGQGTLVTVSSGGSEGKSSGSGSESKSTGGSDIQMTQSPSSLSASVGDRVTITCRASQSISSYLNWYQQKPGEAPKLLIYSASVLQSGVPSRFSGSGSGTDFTLTISSLQPEDFATYYCQQSVMIPMTFGQGTKVEIK

SEQ ID NO: 15 - protein, 16 aa, Artificial Sequence
  Cancer Cell-penetrating functional peptide
GGGGSHRRCNKNNKKR

SEQ ID NO: 16 - protein, 16 aa, Artificial Sequence
  Cancer Cell-penetrating functional peptide
GGGGSHRRCNPNNKKR

SEQ ID NO: 17 - protein, 19 aa, Artificial Sequence
  Cancer Cell-penetrating functional peptide
GGGGSVSRRRRRRGGRRRR

SEQ ID NO: 18 - protein, 20 aa, Artificial Sequence
  Cancer Cell-penetrating functional peptide
GGGGSGKCSTRGRKCCRRKK

SEQ ID NO: 19 - protein, 19 aa, Artificial Sequence
  Cancer Cell-penetrating functional peptide
GGGGSNRPDSAQFWLHHRR

SEQ ID NO: 20 - protein, 16 aa, Artificial Sequence
  Cancer Cell-penetrating functional peptide
HRRCNKNNKKRGGGGS

SEQ ID NO: 21 - protein, 16 aa, Artificial Sequence
  Cancer Cell-penetrating functional peptide
HRRCNPNNKKRGGGGS

SEQ ID NO: 22 - protein, 19 aa, Artificial Sequence
  Cancer Cell-penetrating functional peptide
VSRRRRRRGGRRRRGGGGS

SEQ ID NO: 23 - protein, 20 aa, Artificial Sequence
  Cancer Cell-penetrating functional peptide
GKCSTRGRKCCRRKKGGGGS

SEQ ID NO: 24 - protein, 20 aa, Artificial Sequence
  Cancer Cell-penetrating functional peptide
NRPDSAQFWLHHRRRGGGGS